European Patent Specification EP 3 716 948 B1, published November 22, 2023. Title: Novel Analgesic Pharmaceutical Formulations and Uses Thereof. Applicant: Cytogel Pharma, LLC Maione, Theodore E. Maglaris, Constantine Basil. The sequence listing filed with the application follows.

SEQUENCE LISTING (26 sequences)

SEQ ID NO: 1 - protein, 4 aa, Artificial sequence
  peptide
  MISC_FEATURE (4)..(4): Phe-NH2 (phenylalanine amide)
YPWX

SEQ ID NO: 2 - protein, 4 aa, Artificial sequence
  peptide
  MISC_FEATURE (4)..(4): Phe-NH2 (phenylalanine amide)
YPFX

SEQ ID NO: 3 - protein, 4 aa, Artificial sequence
  peptide
YPWF

SEQ ID NO: 4 - protein, 4 aa, Artificial sequence
  peptide
YPFF

SEQ ID NO: 5 - protein, 4 aa, Artificial sequence
  peptide
  MISC_FEATURE (4)..(4): D-Phe-NH2 (D-phenylalanine amide)
YPWX

SEQ ID NO: 6 - protein, 4 aa, Artificial sequence
  peptide
  MISC_FEATURE (4)..(4): D-Phe-NH2 (D-phenylalanine amide)
YPFX

SEQ ID NO: 7 - protein, 4 aa, Artificial sequence
  peptide
  MISC_FEATURE (4)..(4): pNO2-Phe-NH2 (p-nitrophenylalanine amide)
YPWX

SEQ ID NO: 8 - protein, 4 aa, Artificial sequence
  peptide
  MISC_FEATURE (4)..(4): pNO2-Phe-NH2 (p-nitrophenylalanine amide)
YPFX

SEQ ID NO: 9 - protein, 4 aa, Artificial sequence
  peptide
  MISC_FEATURE (3)..(3): N-Me-Phe (N-methyl phenylalanine)
  MISC_FEATURE (4)..(4): Phe-NH2 (phenylalanine amide)
YPXX

SEQ ID NO: 10 - protein, 4 aa, Artificial sequence
  peptide
  MISC_FEATURE (3)..(3): N-Et-Phe (N-ethyl phenylalanine)
  MISC_FEATURE (4)..(4): Phe-NH2 (phenylalanine amide)
YPXX

SEQ ID NO: 11 - protein, 4 aa, Artificial sequence
  peptide
  MISC_FEATURE (3)..(3): N-Me-Phe (N-methyl phenylalanine)
  MISC_FEATURE (4)..(4): D-Phe-NH2 (D-phenylalanine amide)
YPXX

SEQ ID NO: 12 - protein, 4 aa, Artificial sequence
  peptide
  MISC_FEATURE (3)..(3): N-Et-Phe (N-ethyl phenylalanine)
  MISC_FEATURE (4)..(4): D-Phe-NH2 (D-phenylalanine amide)
YPXX

SEQ ID NO: 13 - protein, 4 aa, Artificial sequence
  peptide
  MISC_FEATURE (2)..(2): D-Lys (D-Lysine)
YXWF

SEQ ID NO: 14 - protein, 4 aa, Artificial sequence
  peptide
  MISC_FEATURE (2)..(2): D-Lys (D-Lysine)
YXFF

SEQ ID NO: 15 - protein, 4 aa, Artificial sequence
  peptide
  MISC_FEATURE (2)..(2): D-Orn (D-Ornithine)
YXWF

SEQ ID NO: 16 - protein, 4 aa, Artificial sequence
  peptide
  MISC_FEATURE (2)..(2): D-Orn (D-Ornithine)
YXFF

SEQ ID NO: 17 - protein, 4 aa, Artificial sequence
  peptide
  MISC_FEATURE (2)..(2): D-Lys (D-Lysine)
  MISC_FEATURE (4)..(4): pNO2-Phe (p-nitrophenylalanine)
YXWX

SEQ ID NO: 18 - protein, 4 aa, Artificial sequence
  peptide
  MISC_FEATURE (2)..(2): D-Lys (D-Lysine)
  MISC_FEATURE (4)..(4): pNO2-Phe (p-nitrophenylalanine)
YXFX

SEQ ID NO: 19 - protein, 4 aa, Artificial sequence
  peptide
  MISC_FEATURE (2)..(2): D-Orn (D-Ornithine)
  MISC_FEATURE (4)..(4): pNO2-Phe (p-nitrophenylalanine)
YXWX

SEQ ID NO: 20 - protein, 4 aa, Artificial sequence
  peptide
  MISC_FEATURE (2)..(2): D-Orn (D-Ornithine)
  MISC_FEATURE (4)..(4): pNO2-Phe (p-nitrophenylalanine)
YXFX

SEQ ID NO: 21 - protein, 4 aa, Artificial sequence
  peptide
  MISC_FEATURE (2)..(2): D-Lys (D-Lysine)
  MISC_FEATURE (3)..(3): N-Me-Phe (N-methyl phenylalanine)
YXXF

SEQ ID NO: 22 - protein, 4 aa, Artificial sequence
  peptide
  MISC_FEATURE (2)..(2): D-Orn (D-Ornithine)
  MISC_FEATURE (3)..(3): N-Me-Phe (N-methyl phenylalanine)
YXXF

SEQ ID NO: 23 - protein, 4 aa, Artificial sequence
  peptide
  MISC_FEATURE (2)..(2): D-Lys (D-Lysine)
  MISC_FEATURE (3)..(3): N-Et-Phe (N-ethyl phenylalanine)
YXXF

SEQ ID NO: 24 - protein, 4 aa, Artificial sequence
  peptide
  MISC_FEATURE (2)..(2): D-Orn (D-Ornithine)
  MISC_FEATURE (3)..(3): N-Et-Phe (N-ethyl phenylalanine)
YXXF

SEQ ID NO: 25 - protein, 4 aa, Artificial sequence
  peptide
  MISC_FEATURE (2)..(2): D-Lys (D-Lysine)
  MISC_FEATURE (3)..(3): N-Me-Phe (N-methyl phenylalanine)
  MISC_FEATURE (4)..(4): D-Phe (D-phenylalanine)
YXXX

SEQ ID NO: 26 - protein, 4 aa, Artificial sequence
  peptide
  MISC_FEATURE (2)..(2): D-Lys (D-Lysine)
  MISC_FEATURE (3)..(3): N-Et-Phe (N-ethyl phenylalanine)
  MISC_FEATURE (4)..(4): D-Phe (D-phenylalanine)
YXXX